European Patent Specification EP 3 636 761 B1, published July 31, 2024. Title: CAR-T cells for cancer treatment. Applicant: MIE University. The sequence listing filed with the application follows.

SEQUENCE LISTING (38 sequences)

SEQ ID NO: 1 - protein, 10 aa, Homo sapiens
GVYDGREHTV

SEQ ID NO: 2 - protein, 10 aa, Artificial
  1A
AVYDGREHTV

SEQ ID NO: 3 - protein, 10 aa, Artificial
  2A
GAYDGREHTV

SEQ ID NO: 4 - protein, 10 aa, Artificial
  3A
GVADGREHTV

SEQ ID NO: 5 - protein, 10 aa, Artificial
  4A
GVYAGREHTV

SEQ ID NO: 6 - protein, 10 aa, Artificial
  5A
GVYDAREHTV

SEQ ID NO: 7 - protein, 10 aa, Artificial
  6A
GVYDGAEHTV

SEQ ID NO: 8 - protein, 10 aa, Artificial
  7A
GVYDGRAHTV

SEQ ID NO: 9 - protein, 10 aa, Artificial
  8A
GVYDGREATV

SEQ ID NO: 10 - protein, 10 aa, Artificial
  9A
GVYDGREHAV

SEQ ID NO: 11 - protein, 10 aa, Artificial
  10A
GVYDGREHTA

SEQ ID NO: 12 - protein, 10 aa, Artificial
  2.10A
GAYDGREHTA

SEQ ID NO: 13 - protein, 10 aa, Artificial
  3M
GVMDGREHTV

SEQ ID NO: 14 - protein, 10 aa, Artificial
  3F
GVFDGREHTV

SEQ ID NO: 15 - protein, 10 aa, Artificial
  5F
GVYDFREHTV

SEQ ID NO: 16 - protein, 10 aa, Artificial
  5W
GVYDWREHTV

SEQ ID NO: 17 - protein, 10 aa, Homo sapiens
EVYDGREHSA

SEQ ID NO: 18 - protein, 10 aa, Homo sapiens
GLYDGREHSV

SEQ ID NO: 19 - protein, 10 aa, Homo sapiens
GVYVGKEHMF

SEQ ID NO: 20 - protein, 10 aa, Homo sapiens
GLYDGREHLI

SEQ ID NO: 21 - protein, 10 aa, Homo sapiens
GVYAGREHFL

SEQ ID NO: 22 - protein, 10 aa, Homo sapiens
GVYDGEEHSV

SEQ ID NO: 23 - protein, 10 aa, Homo sapiens
GLYDGIEHFM

SEQ ID NO: 24 - protein, 10 aa, Homo sapiens
GVYAGREHFV

SEQ ID NO: 25 - protein, 10 aa, Homo sapiens
HVYNGRTHQW

SEQ ID NO: 26 - protein, 10 aa, Homo sapiens
RVYDGREILT

SEQ ID NO: 27 - protein, 10 aa, Homo sapiens
GVYSGRAHPK

SEQ ID NO: 28 - protein, 52 aa, Artificial
  MAGE-A4 Long Peptide
NYKRCFPVIFGKASEGVYDGREHTVYGEPRKAETSYVKVLEHVVRVNARVRI

SEQ ID NO: 29 - protein, 9 aa, Homo sapiens
NYKRCFPVI

SEQ ID NO: 30 - protein, 21 aa, Homo sapiens
AETSYVKVLEHVVRVNARVRI

SEQ ID NO: 31 - DNA, 726 bp, Artificial
  MAGE #17
caggtccagctggtacagtctggggctgaggtgaagaagcctgggtcctcggtgaaggtctcctgcaaggcttctggaggcaccttcagcagctatgctatcagctgggtgcgacaggcccctggacaagggcttgagtggatgggagggatcatccctatctttggtacagcaaactacgcacagaagttccagggcagagtcacgattaccgcggacaaatccacgagcacagcctacatggagctgagcagcctgagatctgaggacacggccgtgtattactgtgcgagatccccccggcgggcatatcatgatgcttttgatatctggggccaagggacaatggtcaccgtctcttcaggtggaggcggttcaggcggaggtggcagcggcggtggcgggagttcctatgagctgactcagccaccctcgatgtcagtggccccaggaaagacggccagcattacctgtggcggagaccatattggaagtaaaagtgttcactggtaccagcagaagccaggccaggcccctgtactggtcgtctatgatgatagcgaccggccctcagggatccctgagcgattctctggctccaactctgggaacacagccactctgaccatcagcgggacccaggctatggatgaggctgactattactgtctggcgtgggacagcagcactgcgatcttcggcggagggaccaagctgaccgtcctc

SEQ ID NO: 32 - protein, 242 aa, Artificial
  MAGE #17
QVQLVQSGAEVKKPGSSVKVSCKASGGTFSSYAISWVRQAPGQGLEWMGGIIPIFGTANYAQKFQGRVTITADKSTSTAYMELSSLRSEDTAVYYCARSPRRAYHDAFDIWGQGTMVTVSSGGGGSGGGGSGGGGSSYELTQPPSMSVAPGKTASITCGGDHIGSKSVHWYQQKPGQAPVLVVYDDSDRPSGIPERFSGSNSGNTATLTISGTQAMDEADYYCLAWDSSTAIFGGGTKLTVL

SEQ ID NO: 33 - DNA, 363 bp, Artificial
  VH of MAGE #17
caggtccagctggtacagtctggggctgaggtgaagaagcctgggtcctcggtgaaggtctcctgcaaggcttctggaggcaccttcagcagctatgctatcagctgggtgcgacaggcccctggacaagggcttgagtggatgggagggatcatccctatctttggtacagcaaactacgcacagaagttccagggcagagtcacgattaccgcggacaaatccacgagcacagcctacatggagctgagcagcctgagatctgaggacacggccgtgtattactgtgcgagatccccccggcgggcatatcatgatgcttttgatatctggggccaagggacaatggtcaccgtctcttca

SEQ ID NO: 34 - DNA, 51 bp, Artificial
  sc of MAGE#17
ggtggaggcggttcaggcggaggtggcagcggcggtggcgggagttcctat

SEQ ID NO: 35 - DNA, 312 bp, Artificial
  VL of MAGE#17
gagctgactcagccaccctcgatgtcagtggccccaggaaagacggccagcattacctgtggcggagaccatattggaagtaaaagtgttcactggtaccagcagaagccaggccaggcccctgtactggtcgtctatgatgatagcgaccggccctcagggatccctgagcgattctctggctccaactctgggaacacagccactctgaccatcagcgggacccaggctatggatgaggctgactattactgtctggcgtgggacagcagcactgcgatcttcggcggagggaccaagctgaccgtcctc

SEQ ID NO: 36 - protein, 121 aa, Artificial
  VH of MAGE#17
QVQLVQSGAEVKKPGSSVKVSCKASGGTFSSYAISWVRQAPGQGLEWMGGIIPIFGTANYAQKFQGRVTITADKSTSTAYMELSSLRSEDTAVYYCARSPRRAYHDAFDIWGQGTMVTVSS

SEQ ID NO: 37 - protein, 17 aa, Artificial
  sc of MAGE#17
GGGGSGGGGSGGGGSSY

SEQ ID NO: 38 - protein, 104 aa, Artificial
  VL of MAGE#17
ELTQPPSMSVAPGKTASITCGGDHIGSKSVHWYQQKPGQAPVLVVYDDSDRPSGIPERFSGSNSGNTATLTISGTQAMDEADYYCLAWDSSTAIFGGGTKLTVL